European Patent Application EP 4 324 478 A2, published February 21, 2024. Title: EPITOPE MIMICS. Applicant: ioGenetics, LLC. Application US, filed February 16, 2023. The sequence listing filed with the application follows.

SEQUENCE LISTING (268 sequences)

SEQ ID NO: 1 - protein, 5 aa, Ebolavirus
DPETN

SEQ ID NO: 2 - protein, 5 aa, Ebolavirus
TPPAT

SEQ ID NO: 3 - protein, 5 aa, Ebolavirus
TGPDN

SEQ ID NO: 4 - protein, 5 aa, Ebolavirus
DSTAS

SEQ ID NO: 5 - protein, 5 aa, Ebolavirus
TSSDP

SEQ ID NO: 6 - protein, 5 aa, Ebolavirus
ESASS

SEQ ID NO: 7 - protein, 5 aa, Ebolavirus
SASSG

SEQ ID NO: 8 - protein, 5 aa, Ebolavirus
TTTSP

SEQ ID NO: 9 - protein, 5 aa, Ebolavirus
ATTAA

SEQ ID NO: 10 - protein, 5 aa, Ebolavirus
NATED

SEQ ID NO: 11 - protein, 5 aa, Ebolavirus
TTAAG

SEQ ID NO: 12 - protein, 5 aa, Ebolavirus
ATTTS

SEQ ID NO: 13 - protein, 5 aa, Ebolavirus
TAAGP

SEQ ID NO: 14 - protein, 5 aa, Ebolavirus
VSNGP

SEQ ID NO: 15 - protein, 5 aa, Ebolavirus
SADSL

SEQ ID NO: 16 - protein, 5 aa, Ebolavirus
AAGPL

SEQ ID NO: 17 - protein, 5 aa, Ebolavirus
IKKPD

SEQ ID NO: 18 - protein, 5 aa, Ebolavirus
GRRTR

SEQ ID NO: 19 - protein, 5 aa, Ebolavirus
KLSST

SEQ ID NO: 20 - protein, 5 aa, Ebolavirus
SENSS

SEQ ID NO: 21 - protein, 5 aa, Ebolavirus
TDVPS

SEQ ID NO: 22 - protein, 5 aa, Ebolavirus
SEATQ

SEQ ID NO: 23 - protein, 5 aa, Ebolavirus
VATDV

SEQ ID NO: 24 - protein, 5 aa, Ebolavirus
LPAAP

SEQ ID NO: 25 - protein, 5 aa, Ebolavirus
ISEAT

SEQ ID NO: 26 - protein, 5 aa, Ebolavirus
ATQVG

SEQ ID NO: 27 - protein, 5 aa, Ebolavirus
QLANE

SEQ ID NO: 28 - protein, 5 aa, Ebolavirus
NATED

SEQ ID NO: 29 - protein, 5 aa, Ebolavirus
IKKPD

SEQ ID NO: 30 - protein, 5 aa, Ebolavirus
KLSST

SEQ ID NO: 31 - protein, 5 aa, Ebolavirus
TDVPS

SEQ ID NO: 32 - protein, 5 aa, Ebolavirus
VATDV

SEQ ID NO: 33 - protein, 5 aa, Ebolavirus
LPAAP

SEQ ID NO: 34 - protein, 5 aa, Ebolavirus
KPGPA

SEQ ID NO: 35 - protein, 5 aa, Ebolavirus
PGPAK

SEQ ID NO: 36 - protein, 5 aa, Ebolavirus
GSSTR

SEQ ID NO: 37 - protein, 5 aa, Ebolavirus
STIES

SEQ ID NO: 38 - protein, 5 aa, Ebolavirus
TIESP

SEQ ID NO: 39 - protein, 5 aa, Ebolavirus
SGKKG

SEQ ID NO: 40 - protein, 5 aa, Ebolavirus
TPTGS

SEQ ID NO: 41 - protein, 5 aa, Ebolavirus
KSGKK

SEQ ID NO: 42 - protein, 5 aa, Ebolavirus
VTSKN

SEQ ID NO: 43 - protein, 5 aa, Ebolavirus
IARGG

SEQ ID NO: 44 - protein, 5 aa, Ebolavirus
GSNGA

SEQ ID NO: 45 - protein, 5 aa, Ebolavirus
KNGQP

SEQ ID NO: 46 - protein, 5 aa, Ebolavirus
GKKVT

SEQ ID NO: 47 - protein, 5 aa, Ebolavirus
TCHSP

SEQ ID NO: 48 - protein, 5 aa, Ebolavirus
RLGPG

SEQ ID NO: 49 - protein, 5 aa, Ebolavirus
RLGPG

SEQ ID NO: 50 - protein, 5 aa, Ebolavirus
RLGPG

SEQ ID NO: 51 - protein, 5 aa, Ebolavirus
RLGPG

SEQ ID NO: 52 - protein, 5 aa, Ebolavirus
RLGPG

SEQ ID NO: 53 - protein, 5 aa, Homo sapiens
ALPAP

SEQ ID NO: 54 - protein, 5 aa, Homo sapiens
GLPAP

SEQ ID NO: 55 - protein, 5 aa, Homo sapiens
ISKAK

SEQ ID NO: 56 - protein, 5 aa, Homo sapiens
KALPA

SEQ ID NO: 57 - protein, 5 aa, Homo sapiens
KSTSG

SEQ ID NO: 58 - protein, 5 aa, Homo sapiens
PAPPV

SEQ ID NO: 59 - protein, 5 aa, Homo sapiens
PPKPK

SEQ ID NO: 60 - protein, 5 aa, Homo sapiens
PREEQ

SEQ ID NO: 61 - protein, 5 aa, Homo sapiens
PSREE

SEQ ID NO: 62 - protein, 5 aa, Homo sapiens
RSTSE

SEQ ID NO: 63 - protein, 5 aa, Homo sapiens
SDEQL

SEQ ID NO: 64 - protein, 5 aa, Homo sapiens
SRDEL

SEQ ID NO: 65 - protein, 5 aa, Homo sapiens
SSPKP

SEQ ID NO: 66 - protein, 5 aa, Homo sapiens
STSES

SEQ ID NO: 67 - protein, 5 aa, Homo sapiens
STYSL

SEQ ID NO: 68 - protein, 5 aa, Homo sapiens
TKPRE

SEQ ID NO: 69 - protein, 5 aa, Homo sapiens
APGGG

SEQ ID NO: 70 - protein, 5 aa, Homo sapiens
APGPG

SEQ ID NO: 71 - protein, 5 aa, Homo sapiens
FAPPR

SEQ ID NO: 72 - protein, 5 aa, Homo sapiens
GLAPG

SEQ ID NO: 73 - protein, 5 aa, Homo sapiens
HTTSD

SEQ ID NO: 74 - protein, 5 aa, Homo sapiens
PGPGE

SEQ ID NO: 75 - protein, 5 aa, Homo sapiens
PWHPP

SEQ ID NO: 76 - protein, 5 aa, Homo sapiens
QRHSP

SEQ ID NO: 77 - protein, 5 aa, Homo sapiens
WHPPG

SEQ ID NO: 78 - protein, 5 aa, Homo sapiens
APPAP

SEQ ID NO: 79 - protein, 5 aa, Homo sapiens
ATPAT

SEQ ID NO: 80 - protein, 5 aa, Homo sapiens
ATTPA

SEQ ID NO: 81 - protein, 5 aa, Homo sapiens
PPAPP

SEQ ID NO: 82 - protein, 5 aa, Homo sapiens
TAANS

SEQ ID NO: 83 - protein, 5 aa, Homo sapiens
TTPAP

SEQ ID NO: 84 - protein, 5 aa, Homo sapiens
APLPP

SEQ ID NO: 85 - protein, 5 aa, Homo sapiens
APPPP

SEQ ID NO: 86 - protein, 5 aa, Homo sapiens
CGPEP

SEQ ID NO: 87 - protein, 5 aa, Homo sapiens
DSGGP

SEQ ID NO: 88 - protein, 5 aa, Homo sapiens
DSSTS

SEQ ID NO: 89 - protein, 5 aa, Homo sapiens
GGTAP

SEQ ID NO: 90 - protein, 5 aa, Homo sapiens
GPRRR

SEQ ID NO: 91 - protein, 5 aa, Homo sapiens
KAPPP

SEQ ID NO: 92 - protein, 5 aa, Homo sapiens
PDTEA

SEQ ID NO: 93 - protein, 5 aa, Homo sapiens
PPQPP

SEQ ID NO: 94 - protein, 5 aa, Homo sapiens
PPRAP

SEQ ID NO: 95 - protein, 5 aa, Homo sapiens
PRPPR

SEQ ID NO: 96 - protein, 5 aa, Homo sapiens
PRRRR

SEQ ID NO: 97 - protein, 5 aa, Homo sapiens
QPAGD

SEQ ID NO: 98 - protein, 5 aa, Homo sapiens
RDSGG

SEQ ID NO: 99 - protein, 5 aa, Homo sapiens
RRRRG

SEQ ID NO: 100 - protein, 5 aa, Homo sapiens
SAPLP

SEQ ID NO: 101 - protein, 5 aa, Homo sapiens
SSTSG

SEQ ID NO: 102 - protein, 5 aa, Homo sapiens
AEQRA

SEQ ID NO: 103 - protein, 5 aa, Homo sapiens
AVSSS

SEQ ID NO: 104 - protein, 5 aa, Homo sapiens
DFGRP

SEQ ID NO: 105 - protein, 5 aa, Homo sapiens
DGTTV

SEQ ID NO: 106 - protein, 5 aa, Homo sapiens
GPGPP

SEQ ID NO: 107 - protein, 5 aa, Homo sapiens
GPPSS

SEQ ID NO: 108 - protein, 5 aa, Homo sapiens
GRKGP

SEQ ID NO: 109 - protein, 5 aa, Homo sapiens
HNRTK

SEQ ID NO: 110 - protein, 5 aa, Homo sapiens
KGPGP

SEQ ID NO: 111 - protein, 5 aa, Homo sapiens
LGAAG

SEQ ID NO: 112 - protein, 5 aa, Homo sapiens
NRTKR

SEQ ID NO: 113 - protein, 5 aa, Homo sapiens
PGPPS

SEQ ID NO: 114 - protein, 5 aa, Homo sapiens
QLGED

SEQ ID NO: 115 - protein, 5 aa, Homo sapiens
RKGPG

SEQ ID NO: 116 - protein, 5 aa, Homo sapiens
SNTHS

SEQ ID NO: 117 - protein, 5 aa, Homo sapiens
SQTVS

SEQ ID NO: 118 - protein, 5 aa, Homo sapiens
SQTVS

SEQ ID NO: 119 - protein, 5 aa, Homo sapiens
SRSGS

SEQ ID NO: 120 - protein, 5 aa, Homo sapiens
SSQTV

SEQ ID NO: 121 - protein, 5 aa, Homo sapiens
SSSST

SEQ ID NO: 122 - protein, 5 aa, Homo sapiens
TAAPP

SEQ ID NO: 123 - protein, 5 aa, Homo sapiens
TDSLD

SEQ ID NO: 124 - protein, 5 aa, Homo sapiens
THNRT

SEQ ID NO: 125 - protein, 5 aa, Homo sapiens
VSSSS

SEQ ID NO: 126 - protein, 5 aa, Zika virus
PRAEA

SEQ ID NO: 127 - protein, 5 aa, Zika virus
TESTE

SEQ ID NO: 128 - protein, 5 aa, Zika virus
ESTEN

SEQ ID NO: 129 - protein, 5 aa, Zika virus
KGRLS

SEQ ID NO: 130 - protein, 5 aa, Zika virus
STENS

SEQ ID NO: 131 - protein, 5 aa, Zika virus
AGADT

SEQ ID NO: 132 - protein, 5 aa, Zika virus
QPENL

SEQ ID NO: 133 - protein, 5 aa, Zika virus
LSSGH

SEQ ID NO: 134 - protein, 5 aa, Zika virus
PVITE

SEQ ID NO: 135 - protein, 5 aa, Zika virus
GGALN

SEQ ID NO: 136 - protein, 5 aa, Zika virus
AKVEV

SEQ ID NO: 137 - protein, 5 aa, Zika virus
ATLGG

SEQ ID NO: 138 - protein, 5 aa, Zika virus
MSGGT

SEQ ID NO: 139 - protein, 5 aa, Zika virus
ARRSR

SEQ ID NO: 140 - protein, 5 aa, Zika virus
SDAGK

SEQ ID NO: 141 - protein, 5 aa, Zika virus
GSSTS

SEQ ID NO: 142 - protein, 5 aa, Zika virus
STRKL

SEQ ID NO: 143 - protein, 5 aa, Zika virus
SHSTR

SEQ ID NO: 144 - protein, 5 aa, Zika virus
RSRRA

SEQ ID NO: 145 - protein, 5 aa, Zika virus
KKRRG

SEQ ID NO: 146 - protein, 5 aa, Zika virus
RRGAD

SEQ ID NO: 147 - protein, 5 aa, Zika virus
EKKRR

SEQ ID NO: 148 - protein, 5 aa, Zika virus
ERKRR

SEQ ID NO: 149 - protein, 5 aa, Zika virus
SVGKK

SEQ ID NO: 150 - protein, 5 aa, Dengue virus
GEDAP

SEQ ID NO: 151 - protein, 5 aa, Zika virus
ESTEN

SEQ ID NO: 152 - protein, 5 aa, Zika virus
EGTEN

SEQ ID NO: 153 - protein, 5 aa, Zika virus
ENTEN

SEQ ID NO: 154 - protein, 5 aa, Zika virus
ETTEN

SEQ ID NO: 155 - protein, 5 aa, Zika virus
ESTGN

SEQ ID NO: 156 - protein, 5 aa, Dengue virus
SLRTT

SEQ ID NO: 157 - protein, 5 aa, Dengue virus
ASRAW

SEQ ID NO: 158 - protein, 5 aa, Dengue virus
IDGPS

SEQ ID NO: 159 - protein, 5 aa, Dengue virus
KGKRA

SEQ ID NO: 160 - protein, 5 aa, Dengue virus
IFTPE

SEQ ID NO: 161 - protein, 5 aa, Dengue virus
TTVTG

SEQ ID NO: 162 - protein, 5 aa, Dengue virus
SLAGP

SEQ ID NO: 163 - protein, 5 aa, Dengue virus
SASRA

SEQ ID NO: 164 - protein, 5 aa, Zika virus
PDSPR

SEQ ID NO: 165 - protein, 5 aa, Dengue virus
AGKRS

SEQ ID NO: 166 - protein, 5 aa, Dengue virus
LEQGK

SEQ ID NO: 167 - protein, 5 aa, Dengue virus
KNSTF

SEQ ID NO: 168 - protein, 5 aa, Zika virus
EECPG

SEQ ID NO: 169 - protein, 5 aa, Zika virus
EETCG

SEQ ID NO: 170 - protein, 5 aa, Zika virus
VEETC

SEQ ID NO: 171 - protein, 5 aa, Dengue virus
SSGRL

SEQ ID NO: 172 - protein, 5 aa, Dengue virus
LAGPR

SEQ ID NO: 173 - protein, 5 aa, Homo sapiens
ITEST

SEQ ID NO: 174 - protein, 5 aa, Homo sapiens
TENSK

SEQ ID NO: 175 - protein, 5 aa, Homo sapiens
KGSEL

SEQ ID NO: 176 - protein, 5 aa, Homo sapiens
DSESG

SEQ ID NO: 177 - protein, 5 aa, Homo sapiens
IDKET

SEQ ID NO: 178 - protein, 5 aa, Homo sapiens
DKETS

SEQ ID NO: 179 - protein, 5 aa, Homo sapiens
DTGSS

SEQ ID NO: 180 - protein, 5 aa, Homo sapiens
RLSPA

SEQ ID NO: 181 - protein, 5 aa, Homo sapiens
SGQRE

SEQ ID NO: 182 - protein, 5 aa, Homo sapiens
RSQQG

SEQ ID NO: 183 - protein, 5 aa, Homo sapiens
PGLGD

SEQ ID NO: 184 - protein, 5 aa, Homo sapiens
SGSGG

SEQ ID NO: 185 - protein, 5 aa, Homo sapiens
DVSGP

SEQ ID NO: 186 - protein, 5 aa, Homo sapiens
QSDQS

SEQ ID NO: 187 - protein, 5 aa, Homo sapiens
TAPDT

SEQ ID NO: 188 - protein, 5 aa, Homo sapiens
SENEL

SEQ ID NO: 189 - protein, 5 aa, Homo sapiens
LPTGT

SEQ ID NO: 190 - protein, 5 aa, Homo sapiens
GSDTD

SEQ ID NO: 191 - protein, 5 aa, Homo sapiens
GAPRI

SEQ ID NO: 192 - protein, 5 aa, Homo sapiens
IRGQG

SEQ ID NO: 193 - protein, 5 aa, Homo sapiens
SGGDD

SEQ ID NO: 194 - protein, 5 aa, Homo sapiens
LPPNP

SEQ ID NO: 195 - protein, 5 aa, Homo sapiens
PSRAS

SEQ ID NO: 196 - protein, 5 aa, Homo sapiens
STSET

SEQ ID NO: 197 - protein, 5 aa, Homo sapiens
TSETP

SEQ ID NO: 198 - protein, 5 aa, Homo sapiens
RKSPS

SEQ ID NO: 199 - protein, 5 aa, Homo sapiens
SGPGA

SEQ ID NO: 200 - protein, 5 aa, Homo sapiens
PGAPA

SEQ ID NO: 201 - protein, 5 aa, Homo sapiens
TPESG

SEQ ID NO: 202 - protein, 5 aa, Homo sapiens
GTTIS

SEQ ID NO: 203 - protein, 5 aa, Homo sapiens
SPRSQ

SEQ ID NO: 204 - protein, 5 aa, Homo sapiens
GRTSS

SEQ ID NO: 205 - protein, 5 aa, Homo sapiens
SPGTP

SEQ ID NO: 206 - protein, 5 aa, Homo sapiens
PGTPG

SEQ ID NO: 207 - protein, 5 aa, Homo sapiens
GAAPT

SEQ ID NO: 208 - protein, 5 aa, Homo sapiens
DPKPK

SEQ ID NO: 209 - protein, 5 aa, Homo sapiens
KPKNP

SEQ ID NO: 210 - protein, 5 aa, Homo sapiens
PAGDN

SEQ ID NO: 211 - protein, 5 aa, Homo sapiens
TAPTT

SEQ ID NO: 212 - protein, 5 aa, Homo sapiens
TPPPP

SEQ ID NO: 213 - protein, 5 aa, Homo sapiens
SETAS

SEQ ID NO: 214 - protein, 5 aa, Homo sapiens
SGSPG

SEQ ID NO: 215 - protein, 5 aa, Homo sapiens
SPGSA

SEQ ID NO: 216 - protein, 5 aa, Homo sapiens
AASPE

SEQ ID NO: 217 - protein, 5 aa, Homo sapiens
PASPP

SEQ ID NO: 218 - protein, 5 aa, Homo sapiens
PPTTP

SEQ ID NO: 219 - protein, 5 aa, Homo sapiens
SPPTS

SEQ ID NO: 220 - protein, 5 aa, Homo sapiens
TPDPK

SEQ ID NO: 221 - protein, 5 aa, Homo sapiens
RPTKP

SEQ ID NO: 222 - protein, 5 aa, Homo sapiens
AGPGA

SEQ ID NO: 223 - protein, 5 aa, Homo sapiens
DPSPA

SEQ ID NO: 224 - protein, 5 aa, Homo sapiens
QPPPR

SEQ ID NO: 225 - protein, 5 aa, Homo sapiens
PNATQ

SEQ ID NO: 226 - protein, 5 aa, Homo sapiens
ATQPE

SEQ ID NO: 227 - protein, 5 aa, Homo sapiens
PPAPS

SEQ ID NO: 228 - protein, 5 aa, Homo sapiens
APSAT

SEQ ID NO: 229 - protein, 5 aa, Homo sapiens
PVPTP

SEQ ID NO: 230 - protein, 5 aa, Homo sapiens
LPPPP

SEQ ID NO: 231 - protein, 5 aa, Homo sapiens
PPPPA

SEQ ID NO: 232 - protein, 5 aa, Homo sapiens
PPPAP

SEQ ID NO: 233 - protein, 5 aa, Homo sapiens
KSRAS

SEQ ID NO: 234 - protein, 5 aa, Homo sapiens
SRASG

SEQ ID NO: 235 - protein, 5 aa, Homo sapiens
ASGKG

SEQ ID NO: 236 - protein, 5 aa, Homo sapiens
SDSEG

SEQ ID NO: 237 - protein, 5 aa, Homo sapiens
TGRPS

SEQ ID NO: 238 - protein, 5 aa, Homo sapiens
EEEEE

SEQ ID NO: 239 - protein, 5 aa, Homo sapiens
EEEEG

SEQ ID NO: 240 - protein, 5 aa, Homo sapiens
SPGPA

SEQ ID NO: 241 - protein, 5 aa, Homo sapiens
EKDKP

SEQ ID NO: 242 - protein, 5 aa, Homo sapiens
PKTPP

SEQ ID NO: 243 - protein, 5 aa, Homo sapiens
KTPPT

SEQ ID NO: 244 - protein, 5 aa, Homo sapiens
AQPPP

SEQ ID NO: 245 - protein, 5 aa, Homo sapiens
QPPPA

SEQ ID NO: 246 - protein, 5 aa, Homo sapiens
PPPAV

SEQ ID NO: 247 - protein, 5 aa, Homo sapiens
TPPPR

SEQ ID NO: 248 - protein, 5 aa, Homo sapiens
PPPRP

SEQ ID NO: 249 - protein, 5 aa, Homo sapiens
PPRPP

SEQ ID NO: 250 - protein, 5 aa, Homo sapiens
PGGPR

SEQ ID NO: 251 - protein, 5 aa, Homo sapiens
PEEGT

SEQ ID NO: 252 - protein, 5 aa, Homo sapiens
GAEQG

SEQ ID NO: 253 - protein, 5 aa, Homo sapiens
AAGPT

SEQ ID NO: 254 - protein, 5 aa, Homo sapiens
PKPQP

SEQ ID NO: 255 - protein, 5 aa, Homo sapiens
PQPHG

SEQ ID NO: 256 - protein, 5 aa, Homo sapiens
PPSNA

SEQ ID NO: 257 - protein, 5 aa, Homo sapiens
TPPKS

SEQ ID NO: 258 - protein, 5 aa, Homo sapiens
GLPTP

SEQ ID NO: 259 - protein, 5 aa, Homo sapiens
LPTPP

SEQ ID NO: 260 - protein, 5 aa, Homo sapiens
PTPPV

SEQ ID NO: 261 - protein, 5 aa, Homo sapiens
RGPAP

SEQ ID NO: 262 - protein, 5 aa, Homo sapiens
AAAPG

SEQ ID NO: 263 - protein, 5 aa, Homo sapiens
AAPGR

SEQ ID NO: 264 - protein, 5 aa, Homo sapiens
GSPPG

SEQ ID NO: 265 - protein, 5 aa, Homo sapiens
RYGDS

SEQ ID NO: 266 - protein, 5 aa, Homo sapiens
DSDGE

SEQ ID NO: 267 - protein, 5 aa, Homo sapiens
PHGEP

SEQ ID NO: 268 - protein, 5 aa, Homo sapiens
PPGEE